European Patent Application EP 4 548 931 A1, published May 7, 2025. Title: ANTI-PCSK9 ANTIBODY PREPARATION AND USE THEREOF. Applicant: AD Pharmaceuticals Co., Ltd. The sequence listing filed with the application follows.

SEQUENCE LISTING (10 sequences)

SEQ ID NO: 1 - protein, 8 aa, synthetic construct
GFTFSSYS

SEQ ID NO: 2 - protein, 8 aa, synthetic construct
ISSSSSYI

SEQ ID NO: 3 - protein, 16 aa, synthetic construct
AREYDFWSAYYDAFDV

SEQ ID NO: 4 - protein, 9 aa, synthetic construct
SRNIGGGND

SEQ ID NO: 5 - skipped

SEQ ID NO: 6 - protein, 11 aa, synthetic construct
QSFDGSLSGSV

SEQ ID NO: 7 - DNA, 369 bp, synthetic construct
  source 1..369: mol_type = other DNA
gaggtgcagctggtggagtctggaggaggcctggtgcagcccggaagatctctgagactgagttgcgccgcttcaggattcacctttagctcctacagcatgaactgggtgcggcaggctcctggcaaggggctggagtgggtctccggaatctctagttcaagctcctacattagctatgcagactccgtccagggaaggttcaccatctctcgcgataacggcaagaacagcctgtatctgcagatgaacagcctgcgagcagaggacacagccctgtacttctgtgccagagaatatgacttctggtccgcctattacgacgccttcgatgtctggggacaggggactatggtcactgtctcaagc

SEQ ID NO: 8 - protein, 123 aa, synthetic construct
EVQLVESGGGLVQPGRSLRLSCAASGFTFSSYSMNWVRQAPGKGLEWVSGISSSSSYISYADSVQGRFTISRDNGKNSLYLQMNSLRAEDTALYFCAREYDFWSAYYDAFDVWGQGTMVTVSS

SEQ ID NO: 9 - DNA, 333 bp, synthetic construct
  source 1..333: mol_type = other DNA
cagagcgaactgactcagccaagaagcgtcagtggatcacctggccagagcgtgacaatctcctgcaccggcacaagcaggaacattggcgggggaaatgacgtccactggtaccagcagcatccagggaaggcccccaaactgctgatctccggagtgattgagcggagctccggcgtccccgatagattcagcgggtccaagtctggaaacacagcttctctgactatcagtggcctgcaggcagaggacgaagccgattactattgccagtctttcgacggcagtctgtcagggagcgtgtttggcactgggaccgatgtgaccgtcctg

SEQ ID NO: 10 - protein, 111 aa, synthetic construct
QSELTQPRSVSGSPGQSVTISCTGTSRNIGGGNDVHWYQQHPGKAPKLLISGVIERSSGVPDRFSGSKSGNTASLTISGLQAEDEADYYCQSFDGSLSGSVFGTGTDVTVL